European Patent Specification EP 3 445 774 B1, published May 28, 2025. Title: Stable pseudotyped viral particles and uses thereof. Applicant: GENETHON. The sequence listing filed with the application follows.

SEQUENCE LISTING (31 sequences)

SEQ ID NO: 1 - DNA, 1617 bp, Artificial Sequence
  cDNA of human HERV-W
atggccctcccttatcatatttttctctttactgttcttttaccctctttcactctcactgcaccccctccatgccgctgtatgaccagtagctccccttaccaagagtttctatggagaatgcagcgtcccggaaatattgatgccccatcgtataggagtctttctaagggaacccccaccttcactgcccacacccatatgccccgcaactgctatcactctgccactctttgcatgcatgcaaatactcattattggacaggaaaaatgattaatcctagttgtcctggaggacttggagtcactgtctgttggacttacttcacccaaactggtatgtctgatgggggtggagttcaagatcaggcaagagaaaaacatgtaaaagaagtaatctcccaactcacccgggtacatggcacctctagcccctacaaaggactagatctctcaaaactacatgaaaccctccgtacccatactcgcctggtaagcctatttaataccaccctcactgggctccatgaggtctcggcccaaaaccctactaactgttggatatgcctccccctgaacttcaggccatatgtttcaatccctgtacctgaacaatggaacaacttcagcacagaaataaacaccacttccgttttagtaggacctcttgtttccaatctggaaataacccatacctcaaacctcacctgtgtaaaatttagcaatactacatacacaaccaactcccaatgcatcaggtgggtaactcctcccacacaaatagtctgcctaccctcaggaatattttttgtctgtggtacctcagcctatcgttgtttgaatggctcttcagaatctatgtgcttcctctcattcttagtgccccctatgaccatctacactgaacaagatttatacagttatgtcatatctaagccccgcaacaaaagagtacccattcttccttttgttataggagcaggagtgctaggtgcactaggtactggcattggcggtatcacaacctctactcagttctactacaaactatctcaagaactaaatggggacatggaacgggtcgccgactccctggtcaccttgcaagatcaacttaactccctagcagcagtagtccttcaaaatcgaagagctttagacttgctaaccgctgaaagagggggaacctgtttatttttaggggaagaatgctgttattatgttaatcaatccggaatcgtcactgagaaagttaaagaaattcgagatcgaatacaacgtagagcagaggagcttcgaaacactggaccctggggcctcctcagccaatggatgccctggattctccccttcttaggacctctagcagctataatattgctactcctctttggaccctgtatctttaacctccttgttaactttgtctcttccagaatcgaagctgtaaaactacaaatggagcccaagatgcagtccaagactaagatctaccgcagacccctggaccggcctgctagcccacgatctgatgttaatgacatcaaaggcacccctcctgaggaaatctcagctgcacaacctctactacgccccaattcagcaggaagcagttag

SEQ ID NO: 2 - DNA, 1617 bp, Artificial Sequence
  cDNA of human HERV-FRD
atgggcctgctcctgctggttctcattctcacgccttcactagcagcctaccgccatcctgatttcccgttattggaaaaagctcagcaactgctccaaagtacaggatccccttactccaccaattgctggttatgtactagctcttccactgaaacaccagggacagcttatccagcctcgcccagagaatggacaagcatagaggcggaattacatatttcctatcgatgggaccctaatctgaaaggactgatgaggcctgcaaatagtcttctttcaacagtaaagcaagatttccctgatatccgccagaaacctcccattttcggacccatctttactaatatcaacctaatgggaatagcccctatttgtgttatggccaaaaggaaaaatggaacaaatgtaggcactcttccaagtacagtctgtaatgttactttcactgtagattctaaccaacagacttaccaaacatacacccacaaccaattccgccatcaaccaagattccccaaacctccaaatattacttttcctcagggaactttgctagataaatccagccggttttgccagggacgcccaagctcatgcagtactcgaaacttctggttccggcctgctgattataaccaatgtctgcaaatttccaacctcagctctacagcggaatgggttctattggaccaaactcgaaattctcttttttgggaaaataaaaccaagggagctaaccagagccaaacaccctgcgtccaagtcttagcaggcatgactatagccaccagctacctgggcatatcagcagtctcagaattttttggaacctccctcacccccttatttcatttccatatctctacatgccttaaaactcaaggagccttttatatttgtggccagtcgattcaccaatgcctccccagtaactggactggaacttgtaccataggctatgtaaccccagacatcttcatagcccctggcaatctctctcttccaataccaatctatgggaattccccgttgcccagggtgaggagggcaatccatttcattccccttctcgcgggactcggcattctagctggtacgggaaccggaattgctggaatcacaaaagcttccctcacctatagccagctctcaaaggaaatagccaacaacattgacaccatggctaaagccttaacgaccatgcaagaacaaatcgactctttagcagccgtagtccttcaaaatcgtcgaggactagacatgttaacggcagcacagggaggaatttgtttggccttagatgaaaaatgttgcttttgggtaaatcaatcaggaaaagtacaagacaacatcagacaactcctaaatcaagcctccagtttacgggaacgagccactcagggttggttaaattgggaaggaacttggaaatggttctcttgggttcttccccttacaggcccacttgttagtctcctacttttgctcctttttggtccatgtctcctaaatctaataacccaatttgtctcctctcgccttcaggccataaagctccagacgaatctcagtgcaggacgccatcctcgcaatattcaagagtcacccttctaa

SEQ ID NO: 3 - DNA, 7150 bp, Artificial Sequence
  pcDNA3.1 SYNCYTIN-1
tcgagtctagagggcccgtttaaacccgctgatcagcctcgactgtgccttctagttgccagccatctgttgtttgcccctcccccgtgccttccttgaccctggaaggtgccactcccactgtcctttcctaataaaatgaggaaattgcatcgcattgtctgagtaggtgtcattctattctggggggtggggtggggcaggacagcaagggggaggattgggaagacaatagcaggcatgctggggatgcggtgggctctatggcttctgaggcggaaagaaccagctggggctctagggggtatccccacgcgccctgtagcggcgcattaagcgcggcgggtgtggtggttacgcgcagcgtgaccgctacacttgccagcgccctagcgcccgctcctttcgctttcttcccttcctttctcgccacgttcgccggctttccccgtcaagctctaaatcggggcatccctttagggttccgatttagtgctttacggcacctcgaccccaaaaaacttgattagggtgatggttcacgtagtgggccatcgccctgatagacggtttttcgccctttgacgttggagtccacgttctttaatagtggactcttgttccaaactggaacaacactcaaccctatctcggtctattcttttgatttataagggattttggggatttcggcctattggttaaaaaatgagctgatttaacaaaaatttaacgcgaattaattctgtggaatgtgtgtcagttagggtgtggaaagtccccaggctccccaggcaggcagaagtatgcaaagcatgcatctcaattagtcagcaaccaggtgtggaaagtccccaggctccccagcaggcagaagtatgcaaagcatgcatctcaattagtcagcaaccatagtcccgcccctaactccgcccatcccgcccctaactccgcccagttccgcccattctccgccccatggctgactaattttttttatttatgcagaggccgaggccgcctctgcctctgagctattccagaagtagtgaggaggcttttttggaggcctaggcttttgcaaaaagctcccgggagcttgtatatccattttcggatctgatcagcacgtgatgaaaaagcctgaactcaccgcgacgtctgtcgagaagtttctgatcgaaaagttcgacagcgtctccgacctgatgcagctctcggagggcgaagaatctcgtgctttcagcttcgatgtaggagggcgtggatatgtcctgcgggtaaatagctgcgccgatggtttctacaaagatcgttatgtttatcggcactttgcatcggccgcgctcccgattccggaagtgcttgacattggggaattcagcgagagcctgacctattgcatctcccgccgtgcacagggtgtcacgttgcaagacctgcctgaaaccgaactgcccgctgttctgcagccggtcgcggaggccatggatgcgatcgctgcggccgatcttagccagacgagcgggttcggcccattcggaccgcaaggaatcggtcaatacactacatggcgtgatttcatatgcgcgattgctgatccccatgtgtatcactggcaaactgtgatggacgacaccgtcagtgcgtccgtcgcgcaggctctcgatgagctgatgctttgggccgaggactgccccgaagtccggcacctcgtgcacgcggatttcggctccaacaatgtcctgacggacaatggccgcataacagcggtcattgactggagcgaggcgatgttcggggattcccaatacgaggtcgccaacatcttcttctggaggccgtggttggcttgtatggagcagcagacgcgctacttcgagcggaggcatccggagcttgcaggatcgccgcggctccgggcgtatatgctccgcattggtcttgaccaactctatcagagcttggttgacggcaatttcgatgatgcagcttgggcgcagggtcgatgcgacgcaatcgtccgatccggagccgggactgtcgggcgtacacaaatcgcccgcagaagcgcggccgtctggaccgatggctgtgtagaagtactcgccgatagtggaaaccgacgccccagcactcgtccgagggcaaaggaatagcacgtgctacgagatttcgattccaccgccgccttctatgaaaggttgggcttcggaatcgttttccgggacgccggctggatgatcctccagcgcggggatctcatgctggagttcttcgcccaccccaacttgtttattgcagcttataatggttacaaataaagcaatagcatcacaaatttcacaaataaagcatttttttcactgcattctagttgtggtttgtccaaactcatcaatgtatcttatcatgtctgtataccgtcgacctctagctagagcttggcgtaatcatggtcatagctgtttcctgtgtgaaattgttatccgctcacaattccacacaacatacgagccggaagcataaagtgtaaagcctggggtgcctaatgagtgagctaactcacattaattgcgttgcgctcactgcccgctttccagtcgggaaacctgtcgtgccagctgcattaatgaatcggccaacgcgcggggagaggcggtttgcgtattgggcgctcttccgcttcctcgctcactgactcgctgcgctcggtcgttcggctgcggcgagcggtatcagctcactcaaaggcggtaatacggttatccacagaatcaggggataacgcaggaaagaacatgtgagcaaaaggccagcaaaaggccaggaaccgtaaaaaggccgcgttgctggcgtttttccataggctccgcccccctgacgagcatcacaaaaatcgacgctcaagtcagaggtggcgaaacccgacaggactataaagataccaggcgtttccccctggaagctccctcgtgcgctctcctgttccgaccctgccgcttaccggatacctgtccgcctttctcccttcgggaagcgtggcgctttctcaatgctcacgctgtaggtatctcagttcggtgtaggtcgttcgctccaagctgggctgtgtgcacgaaccccccgttcagcccgaccgctgcgccttatccggtaactatcgtcttgagtccaacccggtaagacacgacttatcgccactggcagcagccactggtaacaggattagcagagcgaggtatgtaggcggtgctacagagttcttgaagtggtggcctaactacggctacactagaaggacagtatttggtatctgcgctctgctgaagccagttaccttcggaaaaagagttggtagctcttgatccggcaaacaaaccaccgctggtagcggtggtttttttgtttgcaagcagcagattacgcgcagaaaaaaaggatctcaagaagatcctttgatcttttctacggggtctgacgctcagtggaacgaaaactcacgttaagggattttggtcatgagattatcaaaaaggatcttcacctagatccttttaaattaaaaatgaagttttaaatcaatctaaagtatatatgagtaaacttggtctgacagttaccaatgcttaatcagtgaggcacctatctcagcgatctgtctatttcgttcatccatagttgcctgactccccgtcgtgtagataactacgatacgggagggcttaccatctggccccagtgctgcaatgataccgcgagacccacgctcaccggctccagatttatcagcaataaaccagccagccggaagggccgagcgcagaagtggtcctgcaactttatccgcctccatccagtctattaattgttgccgggaagctagagtaagtagttcgccagttaatagtttgcgcaacgttgttgccattgctacaggcatcgtggtgtcacgctcgtcgtttggtatggcttcattcagctccggttcccaacgatcaaggcgagttacatgatcccccatgttgtgcaaaaaagcggttagctccttcggtcctccgatcgttgtcagaagtaagttggccgcagtgttatcactcatggttatggcagcactgcataattctcttactgtcatgccatccgtaagatgcttttctgtgactggtgagtactcaaccaagtcattctgagaatagtgtatgcggcgaccgagttgctcttgcccggcgtcaatacgggataataccgcgccacatagcagaactttaaaagtgctcatcattggaaaacgttcttcggggcgaaaactctcaaggatcttaccgctgttgagatccagttcgatgtaacccactcgtgcacccaactgatcttcagcatcttttactttcaccagcgtttctgggtgagcaaaaacaggaaggcaaaatgccgcaaaaaagggaataagggcgacacggaaatgttgaatactcatactcttcctttttcaatattattgaagcatttatcagggttattgtctcatgagcggatacatatttgaatgtatttagaaaaataaacaaataggggttccgcgcacatttccccgaaaagtgccacctgacgtcgacggatcgggagatctcccgatcccctatggtcgactctcagtacaatctgctctgatgccgcatagttaagccagtatctgctccctgcttgtgtgttggaggtcgctgagtagtgcgcgagcaaaatttaagctacaacaaggcaaggcttgaccgacaattgcatgaagaatctgcttagggttaggcgttttgcgctgcttcgcgatgtacgggccagatatacgcgttgacattgattattgactagttattaatagtaatcaattacggggtcattagttcatagcccatatatggagttccgcgttacataacttacggtaaatggcccgcctggctgaccgcccaacgacccccgcccattgacgtcaataatgacgtatgttcccatagtaacgccaatagggactttccattgacgtcaatgggtggactatttacggtaaactgcccacttggcagtacatcaagtgtatcatatgccaagtacgccccctattgacgtcaatgacggtaaatggcccgcctggcattatgcccagtacatgaccttatgggactttcctacttggcagtacatctacgtattagtcatcgctattaccatggtgatgcggttttggcagtacatcaatgggcgtggatagcggtttgactcacggggatttccaagtctccaccccattgacgtcaatgggagtttgttttggcaccaaaatcaacgggactttccaaaatgtcgtaacaactccgccccattgacgcaaatgggcggtaggcgtgtacggtgggaggtctatataagcagagctctctggctaactagagaacccactgcttactggcttatcgaaattaatacgactcactatagggagacccaagctggctagcgtttaaacttaagcttatggccctcccttatcatatttttctctttactgttcttttaccctctttcactctcactgcaccccctccatgccgctgtatgaccagtagctccccttaccaagagtttctatggagaatgcagcgtcccggaaatattgatgccccatcgtataggagtctttctaagggaacccccaccttcactgcccacacccatatgccccgcaactgctatcactctgccactctttgcatgcatgcaaatactcattattggacaggaaaaatgattaatcctagttgtcctggaggacttggagtcactgtctgttggacttacttcacccaaactggtatgtctgatgggggtggagttcaagatcaggcaagagaaaaacatgtaaaagaagtaatctcccaactcacccgggtacatggcacctctagcccctacaaaggactagatctctcaaaactacatgaaaccctccgtacccatactcgcctggtaagcctatttaataccaccctcactgggctccatgaggtctcggcccaaaaccctactaactgttggatatgcctccccctgaacttcaggccatatgtttcaatccctgtacctgaacaatggaacaacttcagcacagaaataaacaccacttccgttttagtaggacctcttgtttccaatctggaaataacccatacctcaaacctcacctgtgtaaaatttagcaatactacatacacaaccaactcccaatgcatcaggtgggtaactcctcccacacaaatagtctgcctaccctcaggaatattttttgtctgtggtacctcagcctatcgttgtttgaatggctcttcagaatctatgtgcttcctctcattcttagtgccccctatgaccatctacactgaacaagatttatacagttatgtcatatctaagccccgcaacaaaagagtacccattcttccttttgttataggagcaggagtgctaggtgcactaggtactggcattggcggtatcacaacctctactcagttctactacaaactatctcaagaactaaatggggacatggaacgggtcgccgactccctggtcaccttgcaagatcaacttaactccctagcagcagtagtccttcaaaatcgaagagctttagacttgctaaccgctgaaagagggggaacctgtttatttttaggggaagaatgctgttattatgttaatcaatccggaatcgtcactgagaaagttaaagaaattcgagatcgaatacaacgtagagcagaggagcttcgaaacactggaccctggggcctcctcagccaatggatgccctggattctccccttcttaggacctctagcagctataatattgctactcctctttggaccctgtatctttaacctccttgttaactttgtctcttccagaatcgaagctgtaaaactacaaatggagcccaagatgcagtccaagactaagatctaccgcagacccctggaccggcctgctagcccacgatctgatgttaatgacatcaaaggcacccctcctgaggaaatctcagctgcacaacctctactacgccccaattcagcaggaagcagttagc

SEQ ID NO: 4 - DNA, 7134 bp, Artificial Sequence
  pcDNA3.1 SYNCYTIN-2
cactcatggttatggcagcactgcataattctcttactgtcatgccatccgtaagatgcttttctgtgactggtgagtactcaaccaagtcattctgagaatagtgtatgcggcgaccgagttgctcttgcccggcgtcaatacgggataataccgcgccacatagcagaactttaaaagtgctcatcattggaaaacgttcttcggggcgaaaactctcaaggatcttaccgctgttgagatccagttcgatgtaacccactcgtgcacccaactgatcttcagcatcttttactttcaccagcgtttctgggtgagcaaaaacaggaaggcaaaatgccgcaaaaaagggaataagggcgacacggaaatgttgaatactcatactcttcctttttcaatattattgaagcatttatcagggttattgtctcatgagcggatacatatttgaatgtatttagaaaaataaacaaataggggttccgcgcacatttccccgaaaagtgccacctgacgtcgacggatcgggagatctcccgatcccctatggtcgactctcagtacaatctgctctgatgccgcatagttaagccagtatctgctccctgcttgtgtgttggaggtcgctgagtagtgcgcgagcaaaatttaagctacaacaaggcaaggcttgaccgacaattgcatgaagaatctgcttagggttaggcgttttgcgctgcttcgcgatgtacgggccagatatacgcgttgacattgattattgactagttattaatagtaatcaattacggggtcattagttcatagcccatatatggagttccgcgttacataacttacggtaaatggcccgcctggctgaccgcccaacgacccccgcccattgacgtcaataatgacgtatgttcccatagtaacgccaatagggactttccattgacgtcaatgggtggactatttacggtaaactgcccacttggcagtacatcaagtgtatcatatgccaagtacgccccctattgacgtcaatgacggtaaatggcccgcctggcattatgcccagtacatgaccttatgggactttcctacttggcagtacatctacgtattagtcatcgctattaccatggtgatgcggttttggcagtacatcaatgggcgtggatagcggtttgactcacggggatttccaagtctccaccccattgacgtcaatgggagtttgttttggcaccaaaatcaacgggactttccaaaatgtcgtaacaactccgccccattgacgcaaatgggcggtaggcgtgtacggtgggaggtctatataagcagagctctctggctaactagagaacccactgcttactggcttatcgaaattaatacgactcactatagggagacccaagctggctagcatgggcctgctcctgctggttctcattctcacgccttcactagcagcctaccgccatcctgatttcccgttattggaaaaagctcagcaactgctccaaagtacaggatccccttactccaccaattgctggttatgtactagctcttccactgaaacaccagggacagcttatccagcctcgcccagagaatggacaagcatagaggcggaattacatatttcctatcgatgggaccctaatctgaaaggactgatgaggcctgcaaatagtcttctttcaacagtaaagcaagatttccctgatatccgccagaaacctcccattttcggacccatctttactaatatcaacctaatgggaatagcccctatttgtgttatggccaaaaggaaaaatggaacaaatgtaggcactcttccaagtacagtctgtaatgttactttcactgtagattctaaccaacagacttaccaaacatacacccacaaccaattccgccatcaaccaagattccccaaacctccaaatattacttttcctcagggaactttgctagataaatccagccggttttgccagggacgcccaagctcatgcagtactcgaaacttctggttccggcctgctgattataaccaatgtctgcaaatttccaacctcagctctacagcggaatgggttctattggaccaaactcgaaattctcttttttgggaaaataaaaccaagggagctaaccagagccaaacaccctgcgtccaagtcttagcaggcatgactatagccaccagctacctgggcatatcagcagtctcagaattttttggaacctccctcacccccttatttcatttccatatctctacatgccttaaaactcaaggagccttttatatttgtggccagtcgattcaccaatgcctccccagtaactggactggaacttgtaccataggctatgtaaccccagacatcttcatagcccctggcaatctctctcttccaataccaatctatgggaattccccgttgcccagggtgaggagggcaatccatttcattccccttctcgcgggactcggcattctagctggtacgggaaccggaattgctggaatcacaaaagcttccctcacctatagccagctctcaaaggaaatagccaacaacattgacaccatggctaaagccttaacgaccatgcaagaacaaatcgactctttagcagccgtagtccttcaaaatcgtcgaggactagacatgttaacggcagcacagggaggaatttgtttggccttagatgaaaaatgttgcttttgggtaaatcaatcaggaaaagtacaagacaacatcagacaactcctaaatcaagcctccagtttacgggaacgagccactcagggttggttaaattgggaaggaacttggaaatggttctcttgggttcttccccttacaggcccacttgttagtctcctacttttgctcctttttggtccatgtctcctaaatctaataacccaatttgtctcctctcgccttcaggccataaagctccagacgaatctcagtgcaggacgccatcctcgcaatattcaagagtcacccttctaactcgagtctagagggcccgtttaaacccgctgatcagcctcgactgtgccttctagttgccagccatctgttgtttgcccctcccccgtgccttccttgaccctggaaggtgccactcccactgtcctttcctaataaaatgaggaaattgcatcgcattgtctgagtaggtgtcattctattctggggggtggggtggggcaggacagcaagggggaggattgggaagacaatagcaggcatgctggggatgcggtgggctctatggcttctgaggcggaaagaaccagctggggctctagggggtatccccacgcgccctgtagcggcgcattaagcgcggcgggtgtggtggttacgcgcagcgtgaccgctacacttgccagcgccctagcgcccgctcctttcgctttcttcccttcctttctcgccacgttcgccggctttccccgtcaagctctaaatcggggcatccctttagggttccgatttagtgctttacggcacctcgaccccaaaaaacttgattagggtgatggttcacgtagtgggccatcgccctgatagacggtttttcgccctttgacgttggagtccacgttctttaatagtggactcttgttccaaactggaacaacactcaaccctatctcggtctattcttttgatttataagggattttggggatttcggcctattggttaaaaaatgagctgatttaacaaaaatttaacgcgaattaattctgtggaatgtgtgtcagttagggtgtggaaagtccccaggctccccaggcaggcagaagtatgcaaagcatgcatctcaattagtcagcaaccaggtgtggaaagtccccaggctccccagcaggcagaagtatgcaaagcatgcatctcaattagtcagcaaccatagtcccgcccctaactccgcccatcccgcccctaactccgcccagttccgcccattctccgccccatggctgactaattttttttatttatgcagaggccgaggccgcctctgcctctgagctattccagaagtagtgaggaggcttttttggaggcctaggcttttgcaaaaagctcccgggagcttgtatatccattttcggatctgatcagcacgtgatgaaaaagcctgaactcaccgcgacgtctgtcgagaagtttctgatcgaaaagttcgacagcgtctccgacctgatgcagctctcggagggcgaagaatctcgtgctttcagcttcgatgtaggagggcgtggatatgtcctgcgggtaaatagctgcgccgatggtttctacaaagatcgttatgtttatcggcactttgcatcggccgcgctcccgattccggaagtgcttgacattggggaattcagcgagagcctgacctattgcatctcccgccgtgcacagggtgtcacgttgcaagacctgcctgaaaccgaactgcccgctgttctgcagccggtcgcggaggccatggatgcgatcgctgcggccgatcttagccagacgagcgggttcggcccattcggaccgcaaggaatcggtcaatacactacatggcgtgatttcatatgcgcgattgctgatccccatgtgtatcactggcaaactgtgatggacgacaccgtcagtgcgtccgtcgcgcaggctctcgatgagctgatgctttgggccgaggactgccccgaagtccggcacctcgtgcacgcggatttcggctccaacaatgtcctgacggacaatggccgcataacagcggtcattgactggagcgaggcgatgttcggggattcccaatacgaggtcgccaacatcttcttctggaggccgtggttggcttgtatggagcagcagacgcgctacttcgagcggaggcatccggagcttgcaggatcgccgcggctccgggcgtatatgctccgcattggtcttgaccaactctatcagagcttggttgacggcaatttcgatgatgcagcttgggcgcagggtcgatgcgacgcaatcgtccgatccggagccgggactgtcgggcgtacacaaatcgcccgcagaagcgcggccgtctggaccgatggctgtgtagaagtactcgccgatagtggaaaccgacgccccagcactcgtccgagggcaaaggaatagcacgtgctacgagatttcgattccaccgccgccttctatgaaaggttgggcttcggaatcgttttccgggacgccggctggatgatcctccagcgcggggatctcatgctggagttcttcgcccaccccaacttgtttattgcagcttataatggttacaaataaagcaatagcatcacaaatttcacaaataaagcatttttttcactgcattctagttgtggtttgtccaaactcatcaatgtatcttatcatgtctgtataccgtcgacctctagctagagcttggcgtaatcatggtcatagctgtttcctgtgtgaaattgttatccgctcacaattccacacaacatacgagccggaagcataaagtgtaaagcctggggtgcctaatgagtgagctaactcacattaattgcgttgcgctcactgcccgctttccagtcgggaaacctgtcgtgccagctgcattaatgaatcggccaacgcgcggggagaggcggtttgcgtattgggcgctcttccgcttcctcgctcactgactcgctgcgctcggtcgttcggctgcggcgagcggtatcagctcactcaaaggcggtaatacggttatccacagaatcaggggataacgcaggaaagaacatgtgagcaaaaggccagcaaaaggccaggaaccgtaaaaaggccgcgttgctggcgtttttccataggctccgcccccctgacgagcatcacaaaaatcgacgctcaagtcagaggtggcgaaacccgacaggactataaagataccaggcgtttccccctggaagctccctcgtgcgctctcctgttccgaccctgccgcttaccggatacctgtccgcctttctcccttcgggaagcgtggcgctttctcaatgctcacgctgtaggtatctcagttcggtgtaggtcgttcgctccaagctgggctgtgtgcacgaaccccccgttcagcccgaccgctgcgccttatccggtaactatcgtcttgagtccaacccggtaagacacgacttatcgccactggcagcagccactggtaacaggattagcagagcgaggtatgtaggcggtgctacagagttcttgaagtggtggcctaactacggctacactagaaggacagtatttggtatctgcgctctgctgaagccagttaccttcggaaaaagagttggtagctcttgatccggcaaacaaaccaccgctggtagcggtggtttttttgtttgcaagcagcagattacgcgcagaaaaaaaggatctcaagaagatcctttgatcttttctacggggtctgacgctcagtggaacgaaaactcacgttaagggattttggtcatgagattatcaaaaaggatcttcacctagatccttttaaattaaaaatgaagttttaaatcaatctaaagtatatatgagtaaacttggtctgacagttaccaatgcttaatcagtgaggcacctatctcagcgatctgtctatttcgttcatccatagttgcctgactccccgtcgtgtagataactacgatacgggagggcttaccatctggccccagtgctgcaatgataccgcgagacccacgctcaccggctccagatttatcagcaataaaccagccagccggaagggccgagcgcagaagtggtcctgcaactttatccgcctccatccagtctattaattgttgccgggaagctagagtaagtagttcgccagttaatagtttgcgcaacgttgttgccattgctacaggcatcgtggtgtcacgctcgtcgtttggtatggcttcattcagctccggttcccaacgatcaaggcgagttacatgatcccccatgttgtgcaaaaaagcggttagctccttcggtcctccgatcgttgtcagaagtaagttggccgcagtgttat

SEQ ID NO: 5 - protein, 26 aa, Artificial Sequence
  LAH4
KKALLALALHHLAHLALHLALALKKA

SEQ ID NO: 6 - protein, 26 aa, Artificial Sequence
  LAH4-L1
KKALLAHALHLLALLALHLAHALKKA

SEQ ID NO: 7 - protein, 24 aa, Artificial Sequence
  LAH4-L1-dKC
KKALLAHALHLLALLALHLAHALA

SEQ ID NO: 8 - protein, 26 aa, Artificial Sequence
  LAH4-L1-R
RRALLAHALHLLALLALHLAHALRRA

SEQ ID NO: 9 - protein, 26 aa, Artificial Sequence
  LAH4-L0
KKALLAHALAHLALLALHLALHLKKA

SEQ ID NO: 10 - protein, 26 aa, Artificial Sequence
  LAH4-L2
KKALLALALHHLALLALHLAHALKKA

SEQ ID NO: 11 - protein, 26 aa, Artificial Sequence
  LAH4-L3
KKALLALALHHLALLAHHLALALKKA

SEQ ID NO: 12 - protein, 26 aa, Artificial Sequence
  LAH4-L4iso
KKALLHLALLHAALLAHHLALALKKA

SEQ ID NO: 13 - protein, 26 aa, Artificial Sequence
  LAH4-L5
KKALLHLALLHAALLAHLAALHLKKA

SEQ ID NO: 14 - protein, 26 aa, Artificial Sequence
  LAH4-L6iso
KKALLHLALLLAALHAHLAALHLKKA

SEQ ID NO: 15 - protein, 26 aa, Artificial Sequence
  LAH4-A1
KKALLAHALHLLAALALHLAHLLKKA

SEQ ID NO: 16 - protein, 26 aa, Artificial Sequence
  LAH4-A2
KKALLLAALHHLAALALHLAHLLKKA

SEQ ID NO: 17 - protein, 26 aa, Artificial Sequence
  LAH4-A3
KKALLLAALHHLLALAHHLAALLKKA

SEQ ID NO: 18 - protein, 26 aa, Artificial Sequence
  vectofusin-1
KKALLHAALAHLLALAHHLLALLKKA

SEQ ID NO: 19 - protein, 26 aa, Artificial Sequence
  LAH4-A5
KKALLHALLAHLAALLHALLAHLKKA

SEQ ID NO: 20 - protein, 26 aa, Artificial Sequence
  LAH4-A6iso
KKALLHALLAALLAHLHALLAHLKKA

SEQ ID NO: 21 - protein, 25 aa, Artificial Sequence
  LAH4-A4-K1N
KALLHAALAHLLALAHHLLALLKKA

SEQ ID NO: 22 - protein, 26 aa, Artificial Sequence
  LAH4-A4-K3N
KKKLLHAALAHLLALAHHLLALLKKA

SEQ ID NO: 23 - protein, 24 aa, Artificial Sequence
  LAH4-A4-dKC
KKALLHAALAHLLALAHHLLALLA

SEQ ID NO: 24 - protein, 24 aa, Artificial Sequence
  LAH4-A4-dlaa
KKALLHAALAHLLALAHHLLALLK

SEQ ID NO: 25 - protein, 23 aa, Artificial Sequence
  LAH4-A4-d2aa
KKLLHAALAHLLALAHHLLALLK

SEQ ID NO: 26 - protein, 23 aa, Artificial Sequence
  LAH4-A4-d2Caa
KKALLHAALAHLLALAHHLLALK

SEQ ID NO: 27 - protein, 22 aa, Artificial Sequence
  LAH4-A4-d3aa
KKLHAALAHLLALAHHLLALLK

SEQ ID NO: 28 - protein, 20 aa, Artificial Sequence
  LAH4-A4-d5aa
KKLHAALAHLLALAHHLLAK

SEQ ID NO: 29 - protein, 26 aa, Artificial Sequence
  LAH2-A6
KKALLHAALAHLLALAAALLALLKKA

SEQ ID NO: 30 - protein, 26 aa, Artificial Sequence
  K2-L10A12-K2
KKALLAAALAALLALAAALLALLKKA

SEQ ID NO: 31 - protein, 26 aa, Artificial Sequence
  LAH4-A4-Leu
KKLLLHALLAHLLALLHHLLALLKKL